European Patent Specification EP 3 959 235 B1, published July 26, 2023. Title: RITUXIMAB-RESISTANT CHIMERIC ANTIGEN RECEPTORS AND USES THEREOF. Applicant: ALLOGENE THERAPEUTICS, INC. The sequence listing filed with the application follows.

SEQUENCE LISTING (41 sequences)

SEQ ID NO: 1 - DNA, 2019 bp, Artificial Sequence
  source: /note="Description of Artificial Sequence: Synthetic polynucleotide"
  source: /note="chimeric antigen receptor"
atgctgaccagcctgctgtgctggatggccctgtgcctgctgggcgccgaccacgccgatgcctgcccctacagcaaccccagcctgtgcagcggaggcggcggcagcgagctgcccacccagggcaccttctccaacgtgtccaccaacgtgagcccagccaagcccaccaccaccgcctgtccttattccaatccttccctgtgtagcggagggggaggcagcccagcccccagacctcccaccccagcccccaccatcgccagccagcctctgagcctgagacccgaggcctgccgcccagccgccggcggcgccgtgcacaccagaggcctggatttcgcctgcgatatctacatctgggccccactggccggcacctgtggcgtgctgctgctgagcctggtgatcaccctgtactgcaaccaccgcaaccgcaggcgcgtgtgcaagtgccccaggcccgtggtgagagccgagggcagaggcagcctgctgacctgcggcgacgtggaggagaacccaggccccatggagaccgacaccctgctgctgtgggtgctgctgctgtgggtgccaggcagcaccggcgaggtgcagctgcagcagagcggacccgagctgatcaagccaggcgccagcgtgaagatgagctgcaaggccagcggctacaccttcaccagctacgtgatgcactgggtgaagcagaagccaggccagggcctggagtggatcggctacatcaacccctacaacgacggcaccaagtacaacgagaagttcaagggcaaggccaccctgaccagcgacaagagcagcagcaccgcctacatggagctgagcagcctgaccagcgaggacagcgccgtgtactactgcgccagaggcacctactactacggcagccgggtgttcgactactggggccagggcaccaccctgaccgtgagctctggcggaggcggctctggcggaggcggctctggcggaggcggcagcgacatcgtgatgacccaggctgcccccagcatccccgtgaccccaggcgagagcgtgagcatcagctgccggagcagcaagagcctgctgaacagcaacggcaacacctacctgtactggttcctgcagcggccaggccagagcccccagctgctgatctaccggatgagcaacctggccagcggcgtgcccgaccggttcagcggcagcggcagcggcaccgccttcaccctgcggatcagccgggtggaggccgaggacgtgggcgtgtactactgcatgcagcacctggagtaccccttcaccttcggagccggcaccaagctggagctgaagcggtcggatcccaccaccaccccagccccacggccacctacccctgccccaaccatcgccagccagcccctgagcctgcggcctgaagcctgcaggcctgccgccggaggagccgtgcacacaaggggcctggacttcgcctgcgacatctatatctgggcccccctggccgggacatgcggggtgctgctgctgtccctggtgattacactgtattgcaaacggggccggaagaagctgctgtacatcttcaagcagcccttcatgcggcccgtgcagaccacccaggaggaggacggctgcagctgccggttccccgaggaagaggaaggcggctgcgagctgcgggtgaagttcagccggagcgccgacgccccagcctaccagcagggccagaaccagctgtacaacgagctgaacctgggacggcgggaggagtacgacgtgctggacaagcggcggggacgggaccccgagatgggcggcaagcctcgccggaagaatccccaggagggcctgtacaacgagctgcagaaggacaagatggccgaggcctacagcgagatcggcatgaagggcgagcggcgccggggcaagggccacgacggcctgtaccagggcctgagcaccgccaccaaggacacctacgacgccctgcacatgcaggccctgccaccccggtga

SEQ ID NO: 2 - DNA, 1488 bp, Artificial Sequence
  source: /note="Description of Artificial Sequence: Synthetic polynucleotide"
  source: /note="chimeric antigen receptor"
atggagaccgacaccctgctgctgtgggtgctgctgctgtgggtgccaggcagcaccggcgaggtgcagctgcagcagagcggacccgagctgatcaagccaggcgccagcgtgaagatgagctgcaaggccagcggctacaccttcaccagctacgtgatgcactgggtgaagcagaagccaggccagggcctggagtggatcggctacatcaacccctacaacgacggcaccaagtacaacgagaagttcaagggcaaggccaccctgaccagcgacaagagcagcagcaccgcctacatggagctgagcagcctgaccagcgaggacagcgccgtgtactactgcgccagaggcacctactactacggcagccgggtgttcgactactggggccagggcaccaccctgaccgtgagctctggcggaggcggctctggcggaggcggctctggcggaggcggcagcgacatcgtgatgacccaggctgcccccagcatccccgtgaccccaggcgagagcgtgagcatcagctgccggagcagcaagagcctgctgaacagcaacggcaacacctacctgtactggttcctgcagcggccaggccagagcccccagctgctgatctaccggatgagcaacctggccagcggcgtgcccgaccggttcagcggcagcggcagcggcaccgccttcaccctgcggatcagccgggtggaggccgaggacgtgggcgtgtactactgcatgcagcacctggagtaccccttcaccttcggagccggcaccaagctggagctgaagcggtcggatcccaccaccaccccagccccacggccacctacccctgccccaaccatcgccagccagcccctgagcctgcggcctgaagcctgcaggcctgccgccggaggagccgtgcacacaaggggcctggacttcgcctgcgacatctatatctgggcccccctggccgggacatgcggggtgctgctgctgtccctggtgattacactgtattgcaaacggggccggaagaagctgctgtacatcttcaagcagcccttcatgcggcccgtgcagaccacccaggaggaggacggctgcagctgccggttccccgaggaagaggaaggcggctgcgagctgcgggtgaagttcagccggagcgccgacgccccagcctaccagcagggccagaaccagctgtacaacgagctgaacctgggacggcgggaggagtacgacgtgctggacaagcggcggggacgggaccccgagatgggcggcaagcctcgccggaagaatccccaggagggcctgtacaacgagctgcagaaggacaagatggccgaggcctacagcgagatcggcatgaagggcgagcggcgccggggcaagggccacgacggcctgtaccagggcctgagcaccgccaccaaggacacctacgacgccctgcacatgcaggccctgccaccccggtga

SEQ ID NO: 3 - DNA, 1488 bp, Artificial Sequence
  source: /note="Description of Artificial Sequence: Synthetic polynucleotide"
  source: /note="chimeric antigen receptor"
atggagacagataccctgctgctgtgggtgctgctgctgtgggtgcctggctccacaggagaggtgcagctgcagcagtctggaccagagctgatcaagcctggagcatccgtgaagatgtcttgcaaggccagcggctatacattcaccagctacgtgatgcactgggtgaagcagaagcctggccagggcctggagtggatcggctatatcaatccatacaacgacggcaccaagtataatgagaagtttaagggcaaggccacactgacctctgataagagctcctctacagcctacatggagctgagctccctgacctctgaggacagcgccgtgtactattgcgccagaggcacatactattacggcagcagggtgttcgattactggggccagggcaccacactgaccgtgtctagcggaggaggaggctccggaggaggaggctctggcggcggcggcagcgacatcgtgatgacacaggcagcaccaagcatcccagtgacccctggcgagagcgtgtccatctcttgtcggtcctctaagtccctgctgaactctaatggcaacacctatctgtactggtttctgcagcggcccggacagtccccacagctgctgatctataggatgagcaacctggcatccggagtgcctgatcgcttcagcggctccggctctggaacagcctttaccctgaggatctctcgggtggaggcagaggacgtgggcgtgtattactgcatgcagcacctggagtaccccttcacatttggcgcaggaaccaagctggagctgaagcggagcgaccccaccacaacccctgcaccacggccccctacaccagcacctaccatcgcatctcagccactgagcctgcggcccgaggcctgtaggcctgcagcaggaggagcagtgcacaccaggggcctggacttcgcctgcgatatctatatctgggcaccactggcaggaacatgtggcgtgctgctgctgagcctggtcatcaccctgtattgcaagagaggcaggaagaagctgctgtacatcttcaagcagccttttatgcggccagtgcagacaacccaggaggaggatggctgctcctgtagattcccagaggaggaggagggaggatgtgagctgcgcgtgaagtttagccggtccgccgacgcaccagcatatcagcagggccagaatcagctgtacaatgagctgaacctgggccggagagaggagtacgacgtgctggataagaggaggggaagggaccccgagatgggaggcaagccacggagaaagaatccccaggagggcctgtataacgagctgcagaaggataagatggccgaggcctacagcgagatcggcatgaagggagagaggcgccggggcaagggacacgacggcctgtatcagggcctgtccacagccaccaaggacacctacgatgccctgcacatgcaggccctgccaccaaggtga

SEQ ID NO: 4 - DNA, 1875 bp, Artificial Sequence
  source: /note="Description of Artificial Sequence: Synthetic polynucleotide"
  source: /note="chimeric antigen receptor"
atgggaacaagcctgctgtgctggatggctctgtgcctgctgggggccgaccacgctgacgcctccgggggggggggctctcctgcccctaggccccctacacctgcaccaaccatcgcatcccagccactgtctctgcgccctgaggcctgccggccagcagcaggaggagcagtgcacacccgcggcctggacttcgcctgcgatatctatatctgggcaccactggcaggcacatgtggcgtgctgctgctgagcctggtcatcaccctgtactgcaatcacaggaaccggagaagggtgtgcaagtgtccccggcctgtggtgagagcagagggaaggggcagcctgctgacatgtggcgacgtggaggagaatccaggccctatggagacagataccctgctgctgtgggtgctgctgctgtgggtgcccggcagcaccggagaggtgcagctgcagcagtccggaccagagctgatcaagcctggagccagcgtgaagatgtcctgtaaggcctctggctatacattcaccagctacgtgatgcactgggtgaagcagaagcctggccagggcctggagtggatcggctatatcaatccatacaacgacggcacaaagtataacgagaagtttaagggcaaggccacactgacctccgataagagctcctctacagcctacatggagctgagctccctgacctctgaggacagcgccgtgtactattgcgccagaggcacatactattacggctctagggtgttcgattactggggccagggcaccacactgaccgtgtctagcggaggaggaggcagcggaggaggaggctccggcggcggcggctctgacatcgtgatgacacaggcagcaccatccatcccagtgacccctggcgagagcgtgtccatctcttgtcggtcctctaagagcctgctgaactccaatggcaacacctatctgtactggtttctgcagcggcccggacagagcccacagctgctgatctataggatgtctaatctggcaagcggcgtgcccgatcgcttcagcggctccggctctggcacagcctttaccctgaggatctcccgcgtggaggcagaggacgtgggcgtgtattactgcatgcagcacctggagtaccccttcacatttggcgcaggcaccaagctggagctgaagcggagcgaccccaccacaacccctgcaccacggccacccacaccagcacctactattgcatcccagccactgagcctgcggcccgaggcctgtaggcctgccgccggcggcgcagtgcacacccggggcctggactttgcctgcgatatctacatctgggcacctctggccggcacatgcggcgtgctgttactgagcctggtcatcaccctgtattgcaagcggggcagaaagaagctgctgtacatcttcaagcagccttttatgcggccagtgcagacaacccaggaggaggatggctgctcctgtagattcccagaggaggaggagggaggatgtgagctgcgcgtgaagtttagccggtccgccgacgcaccagcatatcagcagggccagaaccagctgtacaatgagctgaacctgggccggagagaggagtatgacgtgctggataagagacggggccgggaccccgagatgggaggcaagccacgccggaagaatccccaggagggcctgtataacgagctgcagaaggataagatggccgaggcctacagcgagatcggcatgaagggagagagaaggcgcggcaagggacacgacggcctgtaccagggcctgagcacagcaacaaaagacacctacgacgcactgcacatgcaggctctgccccctcggtaa

SEQ ID NO: 5 - DNA, 1941 bp, Artificial Sequence
  source: /note="Description of Artificial Sequence: Synthetic polynucleotide"
  source: /note="chimeric antigen receptor"
atgggaacctctctgctgtgctggatggctctgtgcctgctgggggccgatcacgctgacgcaagtggcgggggggggtccgaactgcccacacagggcaccttctccaacgtgagcaccaacgtgagctccggcggaggaggcagccctgcaccaaggccccctacaccagcacctaccatcgcatctcagccactgagcctgcgccccgaggcctgccggcctgcagcaggcggcgccgtgcacacccgcggcctggactttgcctgcgatatctatatctgggcacctctggcaggcacatgtggcgtgctgctgctgagcctggtcatcaccctgtactgcaatcacaggaaccggagaagggtgtgcaagtgtccacggcccgtggtgagagcagagggaaggggctccctgctgacatgtggcgacgtggaggagaatcctggcccaatggagacagataccctgctgctgtgggtgctgctgctgtgggtgcccggctccaccggagaggtgcagctgcagcagtctggaccagagctgatcaagccaggagcatccgtgaagatgtcttgtaaggccagcggctatacattcaccagctacgtgatgcactgggtgaagcagaagccaggacagggcctggagtggatcggctatatcaatccttacaacgacggcaccaagtataacgagaagtttaagggcaaggccacactgacctctgataagtctagctccacagcctacatggagctgtctagcctgaccagcgaggactccgccgtgtactattgcgccagaggcacatactattacggcagcagggtgttcgattactggggccagggcaccacactgaccgtgtcctctggaggaggaggctccggaggaggaggctctggcggcggcggcagcgacatcgtgatgacacaggcagcaccttccatcccagtgaccccaggcgagtctgtgagcatctcctgtcggagctccaagtccctgctgaactctaatggcaacacctatctgtactggtttctgcagcggcccggacagtccccacagctgctgatctataggatgagcaatctggcctccggcgtgccagatcgcttctctggcagcggctccggcacagcctttaccctgaggatctctcgcgtggaggcagaggacgtgggcgtgtattactgcatgcagcacctggagtacccattcacatttggcgcaggcaccaagctggagctgaagcggagcgaccccaccacaaccccagcacctcggccacccacaccagcacccaccatcgcatctcagcctctgagcctgcggcccgaggcctgtaggcccgcagcaggaggagcagtgcacacccggggcctggacttcgcctgcgatatctacatctgggcaccactggccggcacatgcggcgtgctgttactgagcctggtcatcaccctgtattgcaagcggggcagaaagaagctgctgtacatcttcaagcagccctttatgcggcctgtgcagacaacccaggaggaggatggctgctcctgtagattccctgaggaggaggagggaggatgtgagctgcgcgtgaagttttctcggagcgccgacgcaccagcatatcagcagggacagaaccagctgtacaatgagctgaacctgggccggagagaggagtatgacgtgctggataagagacggggccgggaccccgagatgggaggcaagcctcgccggaagaatccacaggagggcctgtataacgagctgcagaaggataagatggccgaggcctacagcgagatcggcatgaagggagagagaaggcgcggcaagggacacgacggcctgtaccagggcctgagcacagcaacaaaagacacctacgacgcactgcacatgcaggctctgccaccaagatga

SEQ ID NO: 6 - DNA, 2019 bp, Artificial Sequence
  source: /note="Description of Artificial Sequence: Synthetic polynucleotide"
  source: /note="chimeric antigen receptor"
atggggacctcactgctgtgctggatggctctgtgcctgctgggggccgaccacgctgacgcctgctctggggggggggggggctcatgctccggaggaggaggctctgagctgccaacccagggcacattctccaacgtgagcaccaacgtgtctcctgccaagccaaccacaaccgcatgcagcggcggaggaggaggcagctgttccggcggcggcggcagccctgccccaaggccccctaccccagcacctacaatcgcatctcagcctctgagcctgcgcccagaggcctgtcggcccgcagcaggaggagcagtgcacacccgcggcctggactttgcctgcgatatctatatctgggcaccactggcaggcacctgtggcgtgctgctgctgagcctggtcatcaccctgtactgcaatcacaggaaccggagaagggtgtgcaagtgtccacggcccgtggtgagagcagagggaaggggctctctgctgacctgtggcgacgtggaggagaatcctggccctatggagacagatacactgctgctgtgggtgctgctgctgtgggtgcccggcagcacaggagaggtgcagctgcagcagtccggacctgagctgatcaagccaggcgcctccgtgaagatgtcttgcaaggccagcggctataccttcacaagctacgtgatgcactgggtgaagcagaagccaggccagggcctggagtggatcggctatatcaatccctacaacgacggcaccaagtataacgagaagtttaagggcaaggccaccctgacaagcgataagagctcctctaccgcctacatggagctgagctccctgacaagcgaggactccgccgtgtactattgcgccagaggcacctactattacggctccagggtgttcgattactggggccagggcacaaccctgacagtgtctagcggaggaggaggcagcggaggaggaggctccggcggcggcggctctgacatcgtgatgacccaggcagcaccatccatccctgtgacaccaggcgagtctgtgagcatctcctgtcggtcctctaagtccctgctgaactctaatggcaacacctatctgtactggtttctgcagcggcccggacagtctcctcagctgctgatctataggatgagcaatctggcctccggcgtgcctgatcgcttctctggcagcggctccggcaccgcctttacactgaggatcagccgcgtggaggcagaggacgtgggcgtgtattactgcatgcagcacctggagtaccctttcacctttggcgccggcacaaagctggagctgaagcggagcgaccccacaaccacaccagcacctcggccacccaccccagcaccaacaatcgcatctcagccactgagcctgcggcccgaggcctgtaggccagccgccggcggcgcagtgcacacccggggcctggacttcgcctgcgatatctacatctgggcccctctggccggcacctgcggcgtgctgttactgagcctggtcatcaccctgtattgcaagcggggcagaaagaagctgctgtacatcttcaagcagcccttcatgcggcccgtgcagaccacacaggaggaggatggctgctcctgtagattcccagaggaggaggagggaggatgtgagctgcgcgtgaagttttctcggagcgccgacgcacctgcatatcagcagggacagaaccagctgtacaatgagctgaacctgggccggagagaggagtatgacgtgctggataagagacggggccgggaccccgagatgggaggcaagccccgccggaagaatcctcaggagggcctgtataacgagctgcagaaggataagatggccgaggcctacagcgagatcggcatgaagggagagagaaggcgcggcaagggccacgacggcctgtaccagggcctgtccacagcaacaaaggatacttatgacgctctgcacatgcaggctctgccccctcggtga

SEQ ID NO: 7 - DNA, 2061 bp, Artificial Sequence
  source: /note="Description of Artificial Sequence: Synthetic polynucleotide"
  source: /note="chimeric antigen receptor"
atgggaaccagcctgctgtgctggatggcactgtgcctgctgggagcagaccacgccgatgccgaactgcctactcaggggacattctctaatgtgagcaccaacgtgagctctggaggaggaggctccgagctgccaacccagggcacattctctaatgtgagcacaaacgtgtctcccgccaagcctaccacaaccgccgaactgcctacccagggcacattttccaacgtgtctaccaacgtgtctagcggaggaggaggctcccccgcacctaggccccctaccccagcaccaacaatcgcaagccagcctctgtccctgcgcccagaggcatgcaggccagcagcaggaggagcagtgcacacccgcggcctggactttgcctgcgatatctatatctgggcaccactggcaggaacctgtggcgtgctgctgctgtctctggtcatcaccctgtactgcaatcacagaaaccggagaagggtgtgcaagtgtcctcggccagtggtgagagcagagggaaggggcagcctgctgacctgtggcgacgtggaggagaatcccggccctatggagacagatacactgctgctgtgggtgctgctgctgtgggtgccaggctctacaggagaggtgcagctgcagcagagcggacctgagctgatcaagccaggcgcctctgtgaagatgagctgcaaggcctccggctataccttcacaagctacgtgatgcactgggtgaagcagaagccaggccagggcctggagtggatcggctatatcaatccctacaacgacggcaccaagtataacgagaagtttaagggcaaggccaccctgacatccgataagagctcctctaccgcctacatggagctgagctccctgacatccgaggactctgccgtgtactattgcgccagaggcacctactattacggctctagggtgttcgattactggggccagggcacaaccctgacagtgtctagcggaggaggaggctctggaggaggaggcagcggcggcggaggctccgacatcgtgatgacccaggcagcaccatccatcccagtgacacctggcgagagcgtgtccatctcttgtaggtcctctaagtctctgctgaacagcaatggcaacacctatctgtactggtttctgcagcggcccggacagagccctcagctgctgatctataggatgtccaatctggcctctggagtgcctgatcgcttcagcggctccggctctggaaccgcctttacactgaggatctcccgcgtggaggcagaggacgtgggcgtgtattactgcatgcagcacctggagtaccctttcacctttggcgccggcacaaagctggagctgaagcggagcgaccccacaaccacaccagcaccccggccaccaacccctgcccctacaatcgcaagccagccactgtccctgcggcccgaggcctgtagacctgccgccggcggcgccgtccatacccgcggcctggatttcgcctgcgatatctacatttgggcccctctggccggcacttgcggcgtgctgctgctgagcctggtcatcaccctgtattgcaagcggggcagaaagaagctgctgtacatcttcaagcagcccttcatgcggcccgtgcagaccacacaggaggaggatggctgctcctgtagattcccagaggaggaggagggaggatgtgagctgcgcgtgaagtttagccggtccgccgacgcacctgcatatcagcagggccagaaccagctgtacaatgagctgaacctgggccggagagaggagtacgacgtgctggataagagaaggggacgggaccccgagatgggaggcaagccccgccggaagaatcctcaggagggcctgtataacgagctgcagaaggataagatggccgaggcctacagcgagatcggcatgaagggagagagaaggcgcggcaagggacacgacggcctgtatcagggcctgtccaccgccacaaaggacacctacgatgccctgcacatgcaggccctgcctccaagatga

SEQ ID NO: 8 - protein, 672 aa, Artificial Sequence
  source: /note="Description of Artificial Sequence: Synthetic polypeptide"
  source: /note="chimeric antigen receptor"
MLTSLLCWMALCLLGADHADACPYSNPSLCSGGGGSELPTQGTFSNVSTNVSPAKPTTTACPYSNPSLCSGGGGSPAPRPPTPAPTIASQPLSLRPEACRPAAGGAVHTRGLDFACDIYIWAPLAGTCGVLLLSLVITLYCNHRNRRRVCKCPRPVVRAEGRGSLLTCGDVEENPGPMETDTLLLWVLLLWVPGSTGEVQLQQSGPELIKPGASVKMSCKASGYTFTSYVMHWVKQKPGQGLEWIGYINPYNDGTKYNEKFKGKATLTSDKSSSTAYMELSSLTSEDSAVYYCARGTYYYGSRVFDYWGQGTTLTVSSGGGGSGGGGSGGGGSDIVMTQAAPSIPVTPGESVSISCRSSKSLLNSNGNTYLYWFLQRPGQSPQLLIYRMSNLASGVPDRFSGSGSGTAFTLRISRVEAEDVGVYYCMQHLEYPFTFGAGTKLELKRSDPTTTPAPRPPTPAPTIASQPLSLRPEACRPAAGGAVHTRGLDFACDIYIWAPLAGTCGVLLLSLVITLYCKRGRKKLLYIFKQPFMRPVQTTQEEDGCSCRFPEEEEGGCELRVKFSRSADAPAYQQGQNQLYNELNLGRREEYDVLDKRRGRDPEMGGKPRRKNPQEGLYNELQKDKMAEAYSEIGMKGERRRGKGHDGLYQGLSTATKDTYDALHMQALPPR

SEQ ID NO: 9 - protein, 495 aa, Artificial Sequence
  source: /note="Description of Artificial Sequence: Synthetic polypeptide"
  source: /note="chimeric antigen receptor"
METDTLLLWVLLLWVPGSTGEVQLQQSGPELIKPGASVKMSCKASGYTFTSYVMHWVKQKPGQGLEWIGYINPYNDGTKYNEKFKGKATLTSDKSSSTAYMELSSLTSEDSAVYYCARGTYYYGSRVFDYWGQGTTLTVSSGGGGSGGGGSGGGGSDIVMTQAAPSIPVTPGESVSISCRSSKSLLNSNGNTYLYWFLQRPGQSPQLLIYRMSNLASGVPDRFSGSGSGTAFTLRISRVEAEDVGVYYCMQHLEYPFTFGAGTKLELKRSDPTTTPAPRPPTPAPTIASQPLSLRPEACRPAAGGAVHTRGLDFACDIYIWAPLAGTCGVLLLSLVITLYCKRGRKKLLYIFKQPFMRPVQTTQEEDGCSCRFPEEEEGGCELRVKFSRSADAPAYQQGQNQLYNELNLGRREEYDVLDKRRGRDPEMGGKPRRKNPQEGLYNELQKDKMAEAYSEIGMKGERRRGKGHDGLYQGLSTATKDTYDALHMQALPPR

SEQ ID NO: 10 - protein, 495 aa, Artificial Sequence; identical to SEQ ID NO: 9
  source: /note="Description of Artificial Sequence: Synthetic polypeptide"
  source: /note="chimeric antigen receptor"

SEQ ID NO: 11 - protein, 624 aa, Artificial Sequence
  source: /note="Description of Artificial Sequence: Synthetic polypeptide"
  source: /note="chimeric antigen receptor"
MGTSLLCWMALCLLGADHADASGGGGSPAPRPPTPAPTIASQPLSLRPEACRPAAGGAVHTRGLDFACDIYIWAPLAGTCGVLLLSLVITLYCNHRNRRRVCKCPRPVVRAEGRGSLLTCGDVEENPGPMETDTLLLWVLLLWVPGSTGEVQLQQSGPELIKPGASVKMSCKASGYTFTSYVMHWVKQKPGQGLEWIGYINPYNDGTKYNEKFKGKATLTSDKSSSTAYMELSSLTSEDSAVYYCARGTYYYGSRVFDYWGQGTTLTVSSGGGGSGGGGSGGGGSDIVMTQAAPSIPVTPGESVSISCRSSKSLLNSNGNTYLYWFLQRPGQSPQLLIYRMSNLASGVPDRFSGSGSGTAFTLRISRVEAEDVGVYYCMQHLEYPFTFGAGTKLELKRSDPTTTPAPRPPTPAPTIASQPLSLRPEACRPAAGGAVHTRGLDFACDIYIWAPLAGTCGVLLLSLVITLYCKRGRKKLLYIFKQPFMRPVQTTQEEDGCSCRFPEEEEGGCELRVKFSRSADAPAYQQGQNQLYNELNLGRREEYDVLDKRRGRDPEMGGKPRRKNPQEGLYNELQKDKMAEAYSEIGMKGERRRGKGHDGLYQGLSTATKDTYDALHMQALPPR

SEQ ID NO: 12 - protein, 646 aa, Artificial Sequence
  source: /note="Description of Artificial Sequence: Synthetic polypeptide"
  source: /note="chimeric antigen receptor"
MGTSLLCWMALCLLGADHADASGGGGSELPTQGTFSNVSTNVSSGGGGSPAPRPPTPAPTIASQPLSLRPEACRPAAGGAVHTRGLDFACDIYIWAPLAGTCGVLLLSLVITLYCNHRNRRRVCKCPRPVVRAEGRGSLLTCGDVEENPGPMETDTLLLWVLLLWVPGSTGEVQLQQSGPELIKPGASVKMSCKASGYTFTSYVMHWVKQKPGQGLEWIGYINPYNDGTKYNEKFKGKATLTSDKSSSTAYMELSSLTSEDSAVYYCARGTYYYGSRVFDYWGQGTTLTVSSGGGGSGGGGSGGGGSDIVMTQAAPSIPVTPGESVSISCRSSKSLLNSNGNTYLYWFLQRPGQSPQLLIYRMSNLASGVPDRFSGSGSGTAFTLRISRVEAEDVGVYYCMQHLEYPFTFGAGTKLELKRSDPTTTPAPRPPTPAPTIASQPLSLRPEACRPAAGGAVHTRGLDFACDIYIWAPLAGTCGVLLLSLVITLYCKRGRKKLLYIFKQPFMRPVQTTQEEDGCSCRFPEEEEGGCELRVKFSRSADAPAYQQGQNQLYNELNLGRREEYDVLDKRRGRDPEMGGKPRRKNPQEGLYNELQKDKMAEAYSEIGMKGERRRGKGHDGLYQGLSTATKDTYDALHMQALPPR

SEQ ID NO: 13 - protein, 672 aa, Artificial Sequence
  source: /note="Description of Artificial Sequence: Synthetic polypeptide"
  source: /note="chimeric antigen receptor"
MGTSLLCWMALCLLGADHADACSGGGGGSCSGGGGSELPTQGTFSNVSTNVSPAKPTTTACSGGGGGSCSGGGGSPAPRPPTPAPTIASQPLSLRPEACRPAAGGAVHTRGLDFACDIYIWAPLAGTCGVLLLSLVITLYCNHRNRRRVCKCPRPVVRAEGRGSLLTCGDVEENPGPMETDTLLLWVLLLWVPGSTGEVQLQQSGPELIKPGASVKMSCKASGYTFTSYVMHWVKQKPGQGLEWIGYINPYNDGTKYNEKFKGKATLTSDKSSSTAYMELSSLTSEDSAVYYCARGTYYYGSRVFDYWGQGTTLTVSSGGGGSGGGGSGGGGSDIVMTQAAPSIPVTPGESVSISCRSSKSLLNSNGNTYLYWFLQRPGQSPQLLIYRMSNLASGVPDRFSGSGSGTAFTLRISRVEAEDVGVYYCMQHLEYPFTFGAGTKLELKRSDPTTTPAPRPPTPAPTIASQPLSLRPEACRPAAGGAVHTRGLDFACDIYIWAPLAGTCGVLLLSLVITLYCKRGRKKLLYIFKQPFMRPVQTTQEEDGCSCRFPEEEEGGCELRVKFSRSADAPAYQQGQNQLYNELNLGRREEYDVLDKRRGRDPEMGGKPRRKNPQEGLYNELQKDKMAEAYSEIGMKGERRRGKGHDGLYQGLSTATKDTYDALHMQALPPR

SEQ ID NO: 14 - protein, 686 aa, Artificial Sequence
  source: /note="Description of Artificial Sequence: Synthetic polypeptide"
  source: /note="chimeric antigen receptor"
MGTSLLCWMALCLLGADHADAELPTQGTFSNVSTNVSSGGGGSELPTQGTFSNVSTNVSPAKPTTTAELPTQGTFSNVSTNVSSGGGGSPAPRPPTPAPTIASQPLSLRPEACRPAAGGAVHTRGLDFACDIYIWAPLAGTCGVLLLSLVITLYCNHRNRRRVCKCPRPVVRAEGRGSLLTCGDVEENPGPMETDTLLLWVLLLWVPGSTGEVQLQQSGPELIKPGASVKMSCKASGYTFTSYVMHWVKQKPGQGLEWIGYINPYNDGTKYNEKFKGKATLTSDKSSSTAYMELSSLTSEDSAVYYCARGTYYYGSRVFDYWGQGTTLTVSSGGGGSGGGGSGGGGSDIVMTQAAPSIPVTPGESVSISCRSSKSLLNSNGNTYLYWFLQRPGQSPQLLIYRMSNLASGVPDRFSGSGSGTAFTLRISRVEAEDVGVYYCMQHLEYPFTFGAGTKLELKRSDPTTTPAPRPPTPAPTIASQPLSLRPEACRPAAGGAVHTRGLDFACDIYIWAPLAGTCGVLLLSLVITLYCKRGRKKLLYIFKQPFMRPVQTTQEEDGCSCRFPEEEEGGCELRVKFSRSADAPAYQQGQNQLYNELNLGRREEYDVLDKRRGRDPEMGGKPRRKNPQEGLYNELQKDKMAEAYSEIGMKGERRRGKGHDGLYQGLSTATKDTYDALHMQALPPR

SEQ ID NO: 15 - DNA, 1189 bp, Artificial Sequence
  source: /note="Description of Artificial Sequence: Synthetic polynucleotide"
  source: /note="artificial promoter"
gcgtgaggctccggtgcccgtcagtgggcagagcgcacatcgcccacagtccccgagaagttggggggaggggtcggcaattgaaccggtgcctagagaaggtggcgcggggtaaactgggaaagtgatgtcgtgtactggctccgcctttttcccgagggtgggggagaaccgtatataagtgcagtagtcgccgtgaacgttctttttcgcaacgggtttgccgccagaacacaggtaagtgccgtgtgtggttcccgcgggcctggcctctttacgggttatggcccttgcgtgccttgaattacttccacgcccctggctgcagtacgtgattcttgatcccgagcttcgggttggaagtgggtgggagagttcgaggccttgcgcttaaggagccccttcgcctcgtgcttgagttgaggcctggcctgggcgctggggccgccgcgtgcgaatctggtggcaccttcgcgcctgtctcgctgctttcgataagtctctagccatttaaaatttttgatgacctgctgcgacgctttttttctggcaagatagtcttgtaaatgcgggccaagatctgcacactggtatttcggtttttggggccgcgggcggcgacggggcccgtgcgtcccagcgcacatgttcggcgaggcggggcctgcgagcgcggccaccgagaatcggacgggggtagtctcaagctggccggcctgctctggtgcctggcctcgcgccgccgtgtatcgccccgccctgggcggcaaggctggcccggtcggcaccagttgcgtgagcggaaagatggccgcttcccggccctgctgcagggagctcaaaatggaggacgcggcgctcgggagagcgggcgggtgagtcacccacacaaaggaaaagggcctttccgtcctcagccgtcgcttcatgtgactccacggagtaccgggcgccgtccaggcacctcgattagttctcgagcttttggagtacgtcgtctttaggttggggggaggggttttatgcgatggagtttccccacactgagtgggtggagactgaagttaggccagcttggcacttgatgtaattctccttggaatttgccctttttgagtttggatcttggttcattctcaagcctcagacagtggttcaaagtttttttcttccatttcaggtgtcgtga

SEQ ID NO: 16 - DNA, 237 bp, Artificial Sequence
  source: /note="Description of Artificial Sequence: Synthetic polynucleotide"
  source: /note="promoter"
gcgtgaggctccggtgcccgtcagtgggcagagcgcacatcgcccacagtccccgagaagttggggggaggggtcggcaattgaaccggtgcctagagaaggtggcgcggggtaaactgggaaagtgatgtcgtgtactggctccgcctttttcccgagggtgggggagaaccgtatataagtgcagtagtcgccgtgaacgttctttttcgcaacgggtttgccgccagaacacag

SEQ ID NO: 17 - protein, 464 aa, Artificial Sequence
  source: /note="Description of Artificial Sequence: Synthetic polypeptide"
  source: /note="immunoglobulin gamma 1 heavy chain"
MEWSWIFLFLLSGTAGVHSEVQLQQSGPELIKPGASVKMSCKASGYTFTSYVMHWVKQKPGQGLEWIGYINPYNDGTKYNEKFKGKATLTSDKSSSTAYMELSSLTSEDSAVYYCARGTYYYGSRVFDYWGQGTTLTVSSAKTTPPSVYPLAPGSAAQTNSMVTLGCLVKGYFPEPVTVTWNSGSLSSGVHTFPAVLQSDLYTLSSSVTVPSSTWPSETVTCNVAHPASSTKVDKKIVPRDCGCKPCICTVPEVSSVFIFPPKPKDVLTITLTPKVTCVVVDISKDDPEVQFSWFVDDVEVHTAQTQPREEQFNSTFRSVSELPIMHQDWLNGKEFKCRVNSAAFPAPIEKTISKTKGRPKAPQVYTIPPPKEQMAKDKVSLTCMITDFFPEDITVEWQWNGQPAENYKNTQPIMDTDGSYFVYSKLNVQKSNWEAGNTFTCSVLHEGLHNHHTEKSLSHSPGK

SEQ ID NO: 18 - protein, 239 aa, Artificial Sequence
  source: /note="Description of Artificial Sequence: Synthetic polypeptide"
  source: /note="immunoglobulin kappa light chain"
MRCLAEFLGLLVLWIPGAIGDIVMTQAAPSIPVTPGESVSISCRSSKSLLNSNGNTYLYWFLQRPGQSPQLLIYRMSNLASGVPDRFSGSGSGTAFTLRISRVEAEDVGVYYCMQHLEYPFTFGAGTKLELKRADAAPTVSIFPPSSEQLTSGGASVVCFLNNFYPKDINVKWKIDGSERQNGVLNSWTDQDSKDSTYSMSSTLTLTKDEYERHNSYTCEATHKTSTSPIVKSFNRNEC

SEQ ID NO: 19 - protein, 136 aa, Artificial Sequence
  source: /note="Description of Artificial Sequence: Synthetic polypeptide"
  source: /note="rituximab binding sequence"
CPYSNPSLCSGGGGSELPTQGTFSNVSTNVSPAKPTTTACPYSNPSLCSGGGGSPAPRPPTPAPTIASQPLSLRPEACRPAAGGAVHTRGLDFACDIYIWAPLAGTCGVLLLSLVITLYCNHRNRRRVCKCPRPVV

SEQ ID NO: 20 - protein, 21 aa, Artificial Sequence
  source: /note="Description of Artificial Sequence: Synthetic peptide"
  source: /note="signal peptide"
MGTSLLCWMALCLLGADHADA

SEQ ID NO: 21 - protein, 157 aa, Artificial Sequence
  source: /note="Description of Artificial Sequence: Synthetic polypeptide"
MGTSLLCWMALCLLGADHADACPYSNPSLCSGGGGSELPTQGTFSNVSTNVSPAKPTTTACPYSNPSLCSGGGGSPAPRPPTPAPTIASQPLSLRPEACRPAAGGAVHTRGLDFACDIYIWAPLAGTCGVLLLSLVITLYCNHRNRRRVCKCPRPVV

SEQ ID NO: 22 - protein, 9 aa, Artificial Sequence
  source: /note="Description of Artificial Sequence: Synthetic peptide"
CPYSNPSLC

SEQ ID NO: 23 - protein, 24 aa, Artificial Sequence
  source: /note="Description of Artificial Sequence: Synthetic peptide"
NSELLSLINDMPITNDQKKLMSNN

SEQ ID NO: 24 - protein, 12 aa, Artificial Sequence
  source: /note="Description of Artificial Sequence: Synthetic peptide"
CQFDLSTRRLKC

SEQ ID NO: 25 - protein, 12 aa, Artificial Sequence
  source: /note="Description of Artificial Sequence: Synthetic peptide"
CQYNLSSRALKC

SEQ ID NO: 26 - protein, 12 aa, Artificial Sequence
  source: /note="Description of Artificial Sequence: Synthetic peptide"
CVWQRWQKSYVC

SEQ ID NO: 27 - protein, 12 aa, Artificial Sequence
  source: /note="Description of Artificial Sequence: Synthetic peptide"
CMWDRFSRWYKC

SEQ ID NO: 28 - protein, 25 aa, Artificial Sequence
  source: /note="Description of Artificial Sequence: Synthetic peptide"
SFVLNWYRMSPSNQTDKLAAFPEDR

SEQ ID NO: 29 - protein, 19 aa, Artificial Sequence
  source: /note="Description of Artificial Sequence: Synthetic peptide"
SGTYLCGAISLAPKAQIKE

SEQ ID NO: 30 - protein, 16 aa, Artificial Sequence
  source: /note="Description of Artificial Sequence: Synthetic peptide"
ELPTQGTFSNVSTNVS

SEQ ID NO: 31 - protein, 12 aa, Artificial Sequence
  source: /note="Description of Artificial Sequence: Synthetic peptide"
GQNDTSQTSSPS

SEQ ID NO: 32 - protein, 16 aa, Artificial Sequence
  source: /note="Description of Artificial Sequence: Synthetic peptide"
GLAVSTISSFFPPGYQ

SEQ ID NO: 33 - protein, 45 aa, Artificial Sequence
  source: /note="Description of Artificial Sequence: Synthetic polypeptide"
TTTPAPRPPTPAPTIASQPLSLRPEACRPAAGGAVHTRGLDFACD

SEQ ID NO: 34 - protein, 231 aa, Artificial Sequence
  source: /note="Description of Artificial Sequence: Synthetic polypeptide"
EPKSPDKTHTCPPCPAPPVAGPSVFLFPPKPKDTLMIARTPEVTCVVVDVSHEDPEVKFNWYVDGVEVHNAKTKPREEQYNSTYRVVSVLTVLHQDWLNGKEYKCKVSNKALPAPIEKTISKAKGQPREPQVYTLPPSRDELTKNQVSLTCLVKGFYPSDIAVEWESNGQPENNYKTTPPVLDSDGSFFLYSKLTVDKSRWQQGNVFSCSVMHEALHNHYTQKSLSLSPGK

SEQ ID NO: 35 - protein, 21 aa, Artificial Sequence
  source: /note="Description of Artificial Sequence: Synthetic peptide"
IYIWAPLAGTCGVLLLSLVIT

SEQ ID NO: 36 - protein, 66 aa, Artificial Sequence
  source: /note="Description of Artificial Sequence: Synthetic polypeptide"
TTTPAPRPPTPAPTIASQPLSLRPEACRPAAGGAVHTRGLDFACDIYIWAPLAGTCGVLLLSLVIT

SEQ ID NO: 37 - protein, 42 aa, Artificial Sequence
  source: /note="Description of Artificial Sequence: Synthetic polypeptide"
KRGRKKLLYIFKQPFMRPVQTTQEEDGCSCRFPEEEEGGCEL

SEQ ID NO: 38 - protein, 113 aa, Artificial Sequence
  source: /note="Description of Artificial Sequence: Synthetic polypeptide"
LRVKFSRSADAPAYQQGQNQLYNELNLGRREEYDVLDKRRGRDPEMGGKPRRKNPQEGLYNELQKDKMAEAYSEIGMKGERRRGKGHDGLYQGLSTATKDTYDALHMQALPPR

SEQ ID NO: 39 - DNA, 943 bp, Artificial Sequence
  source: /note="Description of Artificial Sequence: Synthetic polynucleotide"
  source: /note="intron"
gtaagtgccgtgtgtggttcccgcgggcctggcctctttacgggttatggcccttgcgtgccttgaattacttccacgcccctggctgcagtacgtgattcttgatcccgagcttcgggttggaagtgggtgggagagttcgaggccttgcgcttaaggagccccttcgcctcgtgcttgagttgaggcctggcctgggcgctggggccgccgcgtgcgaatctggtggcaccttcgcgcctgtctcgctgctttcgataagtctctagccatttaaaatttttgatgacctgctgcgacgctttttttctggcaagatagtcttgtaaatgcgggccaagatctgcacactggtatttcggtttttggggccgcgggcggcgacggggcccgtgcgtcccagcgcacatgttcggcgaggcggggcctgcgagcgcggccaccgagaatcggacgggggtagtctcaagctggccggcctgctctggtgcctggcctcgcgccgccgtgtatcgccccgccctgggcggcaaggctggcccggtcggcaccagttgcgtgagcggaaagatggccgcttcccggccctgctgcagggagctcaaaatggaggacgcggcgctcgggagagcgggcgggtgagtcacccacacaaaggaaaagggcctttccgtcctcagccgtcgcttcatgtgactccacggagtaccgggcgccgtccaggcacctcgattagttctcgagcttttggagtacgtcgtctttaggttggggggaggggttttatgcgatggagtttccccacactgagtgggtggagactgaagttaggccagcttggcacttgatgtaattctccttggaatttgccctttttgagtttggatcttggttcattctcaagcctcagacagtggttcaaagtttttttcttccatttcag

SEQ ID NO: 40 - protein, 136 aa, Artificial Sequence
  source: /note="Description of Artificial Sequence: Synthetic polypeptide"
  source: /note="mutated rituximab binding sequences"
CSGGGGGSCSGGGGSELPTQGTFSNVSTNVSPAKPTTTACSGGGGGSCSGGGGSPAPRPPTPAPTIASQPLSLRPEACRPAAGGAVHTRGLDFACDIYIWAPLAGTCGVLLLSLVITLYCNHRNRRRVCKCPRPVV

SEQ ID NO: 41 - protein, 25 aa, Artificial Sequence
  source: /note="Description of Artificial Sequence: Synthetic peptide"
  SITE (1)..(25): /note="This sequence may encompass 1-5 'Gly Gly Gly Gly Ser' repeating units"
GGGGSGGGGSGGGGSGGGGSGGGGS